European Patent Application EP 4 692 361 A1, published February 11, 2026. Title: Methods for producing methyl compound. Applicant: Mitsubishi Chemical Corporation. Application WO. The sequence listing filed with the application follows.

SEQUENCE LISTING (13 sequences)

SEQ ID NO: 1 - DNA, 1109 bp, synthetic construct
  source 1..1109: mol_type = other DNA
catatgacaatatcactagaaaatacgactgtaggccagaatccggccggtggccctccgaccggaaaagcaccgctggacatggaaggcttggcgtggattttgtttggtgctagcgcattccaatatctgaatgcagcgtgcgaattgaacctgttcgagttgctggagaacaaaccgggtttgacgaagccacaaatcggtgctgaactgggtctcgctgatcgtgcaaatgacatcctgctgcttggtgccactgcgaccggtatgctgacggtggaagatggtcgctaccagctggcgacggtcctggctgagttgctgaagaccgatgattggcagcgttttaaagataccgtgggttttgaacaatacgtttgctacgagggccagatcgatttcaccgagagcctacgctctaactccaatgttggtctgcgccgcgtgcgcggcagcggtcgtgatctgtatcatcgtttacatgaaaacccgcaaatggaacaggcgttctacaagtacatgcgttcttggtcagaactggcgaaccagcatctggtggaagttctggatctgagcggtacgagcaaactgctggactgtggtggtggcgacgcagttaattcgattgcattggcccaggcgaacccgcacattgaagcgggtattctggagatcccgccaactgcgccactgaccgaaaaaaaaatcgcggaggcaggcttatctgatcgtattaccgtaaagccgggagacatgcacaccgatgaatttccgaccggctatgacaccgtgatgttcgcacaccagctggtcatctggactccggaggagaataccgccttgctgcgtaaagcgtataacgcacttccggaaggcggccgtgttattatctttaactccatgtccaacgacgagggcgacggcccggttgtggccgcgctcgacagcgtttatttcgccgcgctgccggctgaaggtggcatgatttacagctgggctacctacgaggagagcctaacgaaggcgggtttcaacccggagacatttcaacgtatcgacttcccgggttggaccccgcacggcgtgatcatcgcgaccaagtaagatct

SEQ ID NO: 2 - DNA, 4508 bp, synthetic construct
  source 1..4508: mol_type = other DNA
ccatggcacaacagactcctttgtacgaacaacacacgctttgcggcgctcgcatggtggatttccacggctggatgatgccgctgcattacggttcgcaaatcgacgaacatcatgcggtacgtaccgatgccggaatgtttgatgtgtcacatatgaccatcgtcgatcttcgcggcagccgcacccgggagtttctgcgttatctgctggcgaacgatgtggcgaagctcaccaaaagcggcaaagccctttactcggggatgttgaatgcctctggcggtgtgatagatgacctcatcgtctactactttactgaagatttcttccgcctcgttgttaactccgccacccgcgaaaaagacctctcctggattacccaacacgctgaacctttcggcatcgaaattaccgttcgtgatgacctttccatgattgccgtgcaagggccgaatgcgcaggcaaaagctgccacactgtttaatgacgcccagcgtcaggcggtggaagggatgaaaccgttctttggcgtgcaggcgggcgatctgtttattgccaccactggttataccggtgaagcgggctatgaaattgcgctgcccaatgaaaaagcggccgatttctggcgtgcgctggtggaagcgggtgttaagccatgtggcttgggcgcgcgtgacacgctgcgtctggaagcgggcatgaatctttatggtcaggagatggacgaaaccatctctcctttagccgccaacatgggctggaccatcgcctgggaaccggcagatcgtgactttatcggtcgtgaagccctggaagtgcagcgtgagcatggtacagaaaaactggttggtctggtgatgaccgaaaaaggcgtgctgcgtaatgaactgccggtacgctttaccgatgcgcagggcaaccagcatgaaggcattatcaccagcggtactttctccccgacgctgggttacagcattgcgctggcgcgcgtgccggaaggtattggcgaaacggcgattgtgcaaattcgcaaccgtgaaatgccggttaaagtgacaaaacctgtttttgtgcgtaacggcaaagccgtcgcgtgatttacttttttggagattgattgatgagcaacgtaccagcagaactgaaatacagcaaagaacacgaatggctgcgtaaagaagccgacggcacttacaccgttggtattaccgaacatgctcaggagctgttaggcgatatggtgtttgttgacctgccggaagtgggcgcaacggttagcgcgggcgatgactgcgcggttgccgaatcggtaaaagcggcgtcagacatttatgcgccagtaagcggtgaaatcgtggcggtaaacgacgcactgagcgattccccggaactggtgaacagcgaaccgtatgcaggcggctggatctttaaaatcaaagccagcgatgaaagcgaactggaatcactgctggatgcgaccgcatacgaagcattgttagaagacgagtaacggctttattcctcttctgcgggagaggatcagggtgaggaaaatttatgcctcaccctcactctcttcgtaaggagagaggttcacaattcactgcacgtttcaggaaccatcgctcatgacacagacgttaagccagcttgaaaacagcggcgcttttattgaacgccatatcggaccggacgccgcgcaacagcaagaaatgctgaatgccgttggtgcacaatcgttaaacgcgctgaccggccagattgtgccgaaagatattcaacttgcgacaccaccgcaggttggcgcaccggcgaccgaatacgccgcactggcagaactcaaggctattgccagtcgcaataaacgcttcacgtcttacatcggcatgggttacaccgccgtgcagctaccgccggttatcctgcgtaacatgctggaaaatccgggctggtataccgcgtacactccgtatcaacctgaagtctcccagggccgccttgaagcactgctcaacttccagcaggtaacgctggatttgactggactggatatggcctctgcttctcttctggacgaggccaccgctgccgccgaagcaatggcgatggcgaaacgcgtcagcaaactgaaaaatgccaaccgcttcttcgtggcttccgatgtgcatccgcaaacgctggatgtggtccgtactcgtgccgaaacctttggttttgaagtgattgtcgatgacgcgcaaaaagtgctcgaccatcaggacgtcttcggcgtgctgttacagcaggtaggcactaccggtgaaattcacgactacactgcgcttattagcgaactgaaatcacgcaaaattgtggtcagcgttgccgccgatattatggcgctggtgctgttaactgcgccgggtaaacagggcgcggatattgtttttggttcggcgcaacgcttcggcgtgccgatgggctacggtggcccacacgcggcattctttgcggcgaaagatgaatacaaacgctcaatgccgggccgtattatcggtgtatcgaaagatgcagctggcaataccgcgctgcgcatggcgatgcagactcgcgagcaacatatccgccgtgagaaagcgaactccaacatttgtacttcccaggtactgctggcaaacatcgccagcctgtatgccgtttatcacggcccggttggcctgaaacgtatcgctaaccgcattcaccgtctgaccgatatcctggcggcgggcctgcaacaaaaaggtctgaaactgcgccatgcgcactatttcgacaccttgtgtgtggaagtggccgacaaagcgggcgtactgacgcgtgccgaagcggctgaaatcaacctgcgtagcgatattctgaacgcggttgggatcacccttgatgaaacaaccacgcgtgaaaacgtaatgcagcttttcaacgtgctgctgggcgataaccacggcctggacatcgacacgctggacaaagacgtggctcacgacagccgctctatccagcctgcgatgctgcgcgacgacgaaatcctcacccatccggtgtttaatcgctaccacagcgaaaccgaaatgatgcgctatatgcactcgctggagcgtaaagatctggcgctgaatcaggcgatgatcccgctgggttcctgcaccatgaaactgaacgccgccgccgagatgatcccaatcacctggccggaatttgccgaactgcacccgttctgcccgccggagcaggccgaaggttatcagcagatgattgcgcagctggctgactggctggtgaaactgaccggttacgacgccgtttgtatgcagccgaactctggcgcacagggcgaatacgcgggcctgctggcgattcgtcattatcatgaaagccgcaacgaagggcatcgcgatatctgcctgatcccggcttctgcgcacggaactaaccccgcttctgcacatatggcaggaatgcaggtggtggttgtggcgtgtgataaaaacggcaacatcgatctgactgatctgcgcgcgaaagcggaacaggcgggcgataacctctcctgtatcatggtgacttatccttctacccacggcgtgtatgaagaaacgatccgtgaagtgtgtgaagtcgtgcatcagttcggcggtcaggtttaccttgatggcgcgaacatgaacgcccaggttggcatcacctcgccgggctttattggtgcggacgtttcacaccttaacctacataaaactttctgcattccgcacggcggtggtggtccgggtatgggaccgatcggcgtgaaagcgcatttggcaccgtttgtaccgggtcatagcgtggtgcaaatcgaaggcatgttaacccgtcagggcgcggtttctgcggcaccgttcggtagcgcctctatcctgccaatcagctggatgtacatccgcatgatgggcgcagaagggctgaaaaaagcaagccaggtggcaatcctcaacgccaactatattgccagccgcctgcaggatgccttcccggtgctgtataccggtcgcgacggtcgcgtggcgcacgaatgtattctcgatattcgcccgctgaaagaagaaaccggcatcagcgagctggatattgccaagcgcctgatcgactacggtttccacgcgccgacgatgtcgttcccggtggcgggtacgctgatggttgaaccgactgaatctgaaagcaaagtggaactggatcgctttatcgacgcgatgctggctatccgcgcagaaattgaccaggtgaaagccggtgtctggccgctggaagataacccgctggtgaacgcgccgcacattcagagcgaactggtcgccgagtgggcgcatccgtacagccgtgaagttgcggtattcccggcaggtgtggcagacaaatactggccgacagtgaaacgtctggatgatgtttacggcgaccgtaacctgttctgctcctgcgtaccgattagcgaataccagtaaggatcc

SEQ ID NO: 3 - DNA, 1246 bp, synthetic construct
  source 1..1246: mol_type = other DNA
catatgaaaatcggcatcattggtgcaatggaagaagaagttacgctgctgcgtgacaaaatcgaaaaccgtcaaactatcagtctcggcggttgcgaaatctataccggccaactgaatggaaccgaggttgcgcttctgaaatcgggcatcggtaaagtcgctgcggcgctgggtgccactttgctgttggaacactgcaagccagatgtgattattaacaccggttctgccggtggcctggcaccaacgttgaaagtgggcgatatcgttgtctcggacgaagcacgttatcacgacgcggatgtcacggcatttggttatgaatacggtcagttaccaggctgtccggcaggctttaaagctgacgataaactgatcgctgccgctgaggcctgcattgccgaactgaatcttaacgctgtacgtggcctgattgttagcggcgacgctttcatcaacggttctgttggtctggcgaaaatccgccacaacttcccacaggccattgctgtagagatggaagcgacggcaatcgcccatgtctgccacaatttcaacgtcccgtttgttgtcgtacgcgccatctccgacgtggccgatcaacagtctcatcttagcttcgatgagttcctggctgttgccgctaaacagtccagcctgatggttgagtcactggtgcagaaacttgcacatggctaacaattgaaagaggagaaataccatatgccgttgttagatagcttcacagtcgatcatacccggatggaagcgcctgcagttcgggtggcgaaaacaatgaacaccccgcatggcgacgcaatcaccgtgttcgatctgcgcttctgcgtgccgaacaaagaagtgatgccagaaagagggatccataccctggagcacctgtttgctggttttatgcgtaaccatcttaacggtaatggtgtagagattatcgatatctcgccaatgggctgccgcaccggtttttatatgagtctgattggtacgccagatgagcagcgtgttgctgatgcctggaaagcggcaatggaagacgtgctgaaagtgcaggatcagaatcagatcccggaactgaacgtctaccagtgtggcacttaccagatgcactcgttgcaggaagcgcaggatattgcgcgtagcattctggaacgtgacgtacgcatcaacagcaacgaagaactggcactgccgaaagagaagttgcaggaactgcacatctagatct

SEQ ID NO: 4 - DNA, 1418 bp, synthetic construct
  source 1..1418: mol_type = other DNA
catatgtcagcagtaatgacacccgctggatttacggactacaaagttgcagatattaccctcgcggcttggggtcgtagagaactgatcatagcagagtccgaaatgccggcgctgatgggcctgcgtcgcaaatacgccggtcaacagccgctgaagggtgcgaaaatcctgggctgcattcacatgaccattcagactggcgtactgatcgaaacgctagtggccttgggggcggaggtgcgttggtccagctgcaatatctttagcacccaagatcaggcggcggcggctattgcggcagctggcatcccggtttttgcatggaaaggtgaaaccgaggaagaatatgaatggtgtattgagcagaccatcctgaaagatggccaaccgtgggatgcaaatatggttctggacgacggcggtgatctgaccgagatccttcacaagaagtacccgcagatgttggaacgcattcacggtatcaccgaggagaccaccactggcgtgcatcgtctgctggacatgctgaagaacggtactttgaaggtgccggcgatcaatgttaacgacagcgtcaccaaatcgaaaaatgacaacaaatacggctgccgtcacagcttgaatgacgcaattaaacgtggtactgaccatctgttatctggtaagcaagctttagttattggttatggtgatgttggtaaaggttcctctcagagcctccgccaggagggcatgattgttaaggtggcggaagtcgatccgatctgtgcaatgcaagcgtgcatggatggattcgaagtggtgtcgccgtataaaaacggcatcaacgacgggacggaggctagcattgacgctgctctgctgggcaagatcgacttgatcgtgaccacgacgggtaacgtgaatgtgtgtgatgcgaacatgctgaaagccctgaagaagcgggcagttgtgtgcaacatcggccactttgacaatgagatcgataccgcatttatgcgtaagaactgggcgtgggaagaggtcaaaccgcaagtgcacaaaatccatcgcacgggtaaggacggcttcgacgcgcataacgacgattacctgattctgctggcggagggtcgtttagtgaacctgggtaacgcaaccggtcatccgagccgtattatggacggtagctttgccaaccaggttttagcgcagattcacctcttcgagcaaaaatatgcggatctgccagcggcggagaaagccaagcgcttgtcagttgaagttttgcctaagaagctggatgaagaggttgccctggaaatggttaagggcttcggtggcgtagttacccagctgaccccgaaacaagcggagtacatcggcgtcagcgtcgaaggtccattcaagccggatacctatcgttactaagatct

SEQ ID NO: 5 - DNA, 1076 bp, synthetic construct
  source 1..1076: mol_type = other DNA
catatgacagcaactcacaggtcagctaattattccaagccggcgcaactggatatgccgggcttagcgaacttgctgtttggtcatgctgcgttccagtacctgcaagcggcgtgcgaattgaatgtgctggagacagtgcgcaccctgcctgatccgaccaaagagaagctgcgtgaagcgctaggcttagaggagcgtgcagcggatattctgcttcttggcgttaccgcattgggtctgttggttaaagacaacggtgtgtaccacgtggccgatgttgtgcgtgagctgatggataccgatgattggcagagattcaaggacaccgtcgctttcgaacattatatcgtgtacgagggtcagattgacttcaccgaatccctgcaaaaaaacaccaatgttggcttgcgccgttttccgggcgaagggcgcgatatctaccaccgtctgcaccaaaacccgaagctggagaaggtcttttatcgttatatgcgtagctggtcggaactggccaacaaagacctcgtccagcatctggacctgagcaccacccaccgcctgttggacgcgggtggcggtgacgctgtgaacgcactcgcgttggcgcaggcgaacccgaagttagaggtgacggttctggacatcagtcattccattccggttacgcaaagcaaaatcgacgagtctggtctgggtgatcgtgtaaatgcgaaggcgttggacatcctgcacgaaccgttcccaagcggttatgactgtattctgttcgctcaccagctggttatttggacgctggaagagaacacccacatgctgaaaaaagcctatgacgcactgccggaaggtggccgtgtcgtgatttttaattctatgagcaatgatgagggcgatggtccgatcgtggcagcgttggacagcgtttacttcgcgtgcctgccggcagaaggcggaatgatttacgcttgggaacagtacgagcgctgcctggctgaagttggctttaagcatccgcaacgtatccatgttccgggttggactccacatggtattatcatcgcccacaaataagatct

SEQ ID NO: 6 - DNA, 1554 bp, synthetic construct
  source 1..1554: mol_type = other DNA
agatctagaggagaaaactagtatgcctgatatgaagctttttgctggtaacgccaccccggaactagcacaacgtattgccaaccgcctgtacacttcactcggcgacgccgctgtaggtcgctttagcgatggcgaagtcagcgtacaaattaatgaaaatgtacgcggtggtgatattttcatcatccagtccacttgtgcccctactaacgacaacctgatggaattagtcgttatggttgatgccctgcgtcgtgcttccgcaggtcgtatcaccgctgttatcccctactttggctatgcgcgccaggaccgtcgcgtccgttccgctcgtgtaccaatcactgcgaaagtggttgcagacttcctctccagcgtcggtgttgaccgtgtgctgacagtggatctgcacgctgaacagattcagggtttcttcgacgttccggttgataacgtatttggtagcccgatcctgctggaagacatgctgcagctgaatctggataacccaattgtggtttctccggacatcggcggcgttgtgcgtgcccgcgctatcgctaagctgctgaacgataccgatatggcaatcatcgacaaacgtcgtccgcgtgcgaacgtttcacaggtgatgcatatcatcggtgacgttgcaggtcgtgactgcgtactggtcgatgatatgatcgacactggcggtacgctgtgtaaagctgctgaagctctgaaagaacgtggtgctaaacgtgtatttgcgtacgcgactcacccgatcttctctggcaacgcggcgaacaacctgcgtaactctgtaattgatgaagtcgttgtctgcgataccattccgctgagcgatgaaatcaaatcactgccgaacgtgcgtactctgaccctgtcaggtatgctggccgaagcgattcgtcgtatcagcaacgaagaatcgatctctgccatgttcgaacactaaggtaccaaagaggagaaatactagatgaccgcgactgcacagcagcttgagtatctcaaaaatagcatcaaaagcattcaggactacccaaaacccggcattcttttccgcgatgtcaccagcttactggaagacccgaaagcttacgctctcagcatcgacttgctggttgagcgttacaaaaatgcgggcattaccaaagttgtcggcaccgaagcgcgtggcttcttgtttggcgctccggtagctctgggtctgggcgttggctttgtaccggtccgtaaaccgggcaaactgccgcgtgaaaccatcagtgaaacttacgacctggaatacggcaccgatcagctggagatccacgttgatgccatcaaaccgggcgacaaagttctggtggtggacgacctgctggcaaccggcggcactatcgaagcgaccgttaaactgatccgtcgtctgggtggtgaagtggctgacgctgcgttcattatcaacctgttcgatctcggcggcgaacagcgtctcgaaaaacagggcattaccagctacagccttgtcccgttcccgggccattaaggccggcc

SEQ ID NO: 7 - DNA, 1053 bp, synthetic construct
  source 1..1053: mol_type = other DNA
agatctaaagaggagaaatactagatgacagctcccttagttgtactaggaaatccactgttggacttccaagcagatgttacggctgaatacctggcgaagtactctctgaaagaaaacgatgccattttggtggatgcgaagtccggtgatgcaaagatggcgatttttgatgaactgctgcagatgccggaaaccaaactggttgcagggggtgcggctcaaaacaccgctcgcggtgcggcgtatgttctgggcgctggccaagttgtctacttcggctccgttggcaaggacaaatttagtgaacgtttactgaacgagaacgagaaagcaggtgtcaaaagcatgtatcaggttcagaatgacattggtacgggtaagtgcgctgcgcttatcaccggtcataatcgcagcttggtaactgacctgggtgcggcgaacttttttacgcctgaccacctggacaaacattgggatttggtcgaggccgccaagctgttctacatcggcggcttccacctgactgttagcccggacgcgatcgtgaagctcggacaacacgcaaaagagaacagcaaaccgttcgtgctcaattttagcgcaccgtttatcccacatgtttttaaagacgccctggcgcgtgtcctgccgtatgcgaccgtcatcatcgccaacgagagcgaagcggaagcgttctgcgatgctttccagctggactgtgcgaacaccgatttggaagccatcgcgcaacgtattgttaaggactctccggttgagaaaaccgtgattttcacccacggcgtggagccgaccgtggtggtgagctcgaaaggcacctcgacctatccggtgaagccgttggacagctcaaaaatcgtggataccaatggtgcaggcgacgctttcgccggcggttttatggctggcctgaccaagggtgaggatttggagacatctattgatatgggtcagtggctggcagcgctgagcattcaggaggttggtccgtcctacccgtccgaaaagatcagctacagcaagtaacaattg

SEQ ID NO: 8 - DNA, 3405 bp, synthetic construct
  source 1..3405: mol_type = other DNA
ccatggcagcgacagctgctctaaggtcaggagacacccgtgctcaaaccgcggcggcgttcccgccacctccggtgacggctcgccccatcgaccgcgctgcgtggatcgccgcgttccgcttcgtgcgttccgaaactgagcgccgtgctgctccgttgtctgctgaagatcagcaggttcagagcatggcggacgcaagcccgacaaaatggcaccgtgcgcacgtgacgtggttcttcgagcagttcctgctgcgtgagcacctgccgggttacgcaatttatgacgaacgtctgcactacctgtttaactcctattacgtggctgcgggcccgcgtcagccgcgtatccagcgtggcatgattacccgtccgacgatggcggaggtgactgcgtaccgtgcacacgtcgatcgtgccgtcgagtcgctgctggggcaagcggcggacggcgcgttggaagcggtgctgccgatcttggagatcggcttatatcatgaacaacaacatcaagaactgttgttgaccgatatcctccacgccttcgcccaaaacccgctaggcccagtctatgacgcggagtggcgtttcccggcagtggctggccagggtggccaggctccgctggcgagaggtattgcatggattggtcacgagggtgatggtttttcttttgacaacgagtccccgcgtcatgaggccctcattctgcctggacgtatcgataaagcgttggttaccaatcgcgactggctgggctttatggaagccggtggttacgccaagccggaactgtggctgtcagacggctggtatgcgggtcaagcggagggttgggaggcaccgggctactggcgtcgtgatggtgaaggctgggcaaccatgaccctgggtggtgttcgtccggtagagctggatgcaccggtcacgcatattagctactatgaggccgatgcctacgcgcgctgggcaggccgtaccctgccgacggaatttgagtgggaagttgcagctcgcgacggcgcacttccggatgcatttggtcttgtttggcaatggaccagaagcgcgtacgttgcgtacccgggttaccggccactgccgggtgcgctgggcgaatataacggcaagtttatggttagccagttcgtgctgcgtggtagcagcgttgcgaccccggaaggccacgcacgcttgccgtatcgtaattttttttatccgcatcagcgttggcagttcaccggtttgcgcctggcggacgtggcctaaacgcgtagaggagaaatacatcatgacattgtcactagctaattatttagcagcggactctgccgcggaggcgctgcgtcgcgatgttcgtgcgggcttgactgcggctccgaagagcctgccaccaaagtggttttacgacgctgtgggctccgatttgtttgaccagattacccgtctgccggaatattacccgacccgtaccgaagctcaaatcctgcgtaccagaagcgcagagatcatcgcggcggctggtgcagataccctcgtggagctgggcagcggtacgagcgaaaaaacccgcatgctgctggacgctatgcgagacgctgagttgttgcgtcgttttatcccgtttgacgtggatgccggggtgctgcgctctgcgggagcggcgattggcgcagagtacccgggtattgagatcgatgcggtctgtggtgatttcgaagagcacctgggcaaaatcccgcatgttggtcgtcgtttagtagtctttcttggcagtaccattggtaatctgactccggcaccgcgtgcagagttcctgagcaccttggcggacaccctgcagccgggtgactccttgctgttgggtaccgacctggttaaagataccggtcgcctggttcgcgcgtatgatgatgcggcgggcgttaccgcggcgttcaaccgcaacgttctggcggtggtgaaccgtgaattgtcggctgacttcgacttagacgcgttcgagcacgtggccaaatggaacagcgacgaagaacgtattgagatgtggctgcgtgcgcgtacggcccaacacgtgcgtgttgcagcgctggatctggaagtggacttcgcagctggtgaagagatgctcacggaagttagctgcaagtttcgtccggaaaatgttgttgcagagctggctgaggcgggcctgcgccagacccattggtggaccgatccggcaggcgacttcggtctctccctggccgtccgctaaggatccaaagaggagaaaactagtatgatgctagctcagcaatggagggatgcacgtccgaaagtggcgggtctgcacctggactccggtgcatgcagccgtcaaagctttgcggtcatcgacgccacgactgcgcacgcacgccacgaagcagaggtgggcggttatgttgctgcggaggcggctaccccggcgctcgacgctggccgtgcggcggtggcctctctgattggtttcgccgcttccgatgtggtgtacaccagcggtagcaaccacgcgattgatctgctgctgtcttcctggccgggtaagcgcaccctggcgtgtctgccgggtgaatatggccccaacctgagcgcaatggcagcgaatggtttccaggttcgtgcactgccggtggacgacgacggtcgcgtgctggtagacgaagccagccacgagctcagtgcccacccggttgcgttggtgcatcttaccgcgctcgcgtcccatcgtggtatcgcccaaccggcggcggaattggtcgaggcgtgccataacgccggtattccggttgtgatcgatgctgctcaggcacttggtcatctggactgtaatgttggcgctgatgccgtttacagctcgtcccgtaaatggctggcgggtccgcgtggcgttggcgtgctggcggttcgcccggaattggcggagcgcctgcagccgagaatcccaccgtcagattggcctattccgatgagcgttttggagaagctggagttaggtgaacacaacgcagcggcgcgtgtgggcttcagcgttgcggtaggcgagcacctggcggctggtccgaccgccgtgcgcgagcgtttggcggaggtcggccgcctgagccgtcaagttctggcagaagtggacggctggcgtgtggttgaaccggtggaccagccgacggcaatcaccaccttggagagcaccgatggcgccgatccggcttctgttcgtagctggctgatcgcggaacgtggcattgttactacggcctgcgaactggcgcgtgcaccgtttgaaatgcgtaccccggtgttgcgcatcagcccgcatgttgatgttaccgtagacgagctggaacagtttgcagcggctctgagagaagcgccataagaattc

SEQ ID NO: 9 - DNA, 1263 bp, synthetic construct
  source 1..1263: mol_type = other DNA
catatgttaaagcgtgaaatgaacattgccgattatgatgccgaactgtggcaggctatggagcaggaaaaagtacgtcaggaagagcacatcgaactgatcgcctccgaaaactacaccagcccgcgcgtaatgcaggcgcagggttctcagctgaccaacaaatatgctgaaggttatccgggcaaacgctactacggcggttgcgagtatgttgatatcgttgaacaactggcgatcgatcgtgcgaaagaactgttcggcgctgactacgctaacgtccagccgcactccggctcccaggctaactttgcggtctacaccgcgctgctggaaccaggtgataccgttctgggtatgaacctggcgcatggcggtcacctgactcacggttctccggttaacttctccggtaaactgtacaacatcgttccttacggtatcgatgctaccggtcatatcgactacgccgatctggaaaaacaagccaaagaacacaagccgaaaatgattatcggtggtttctctgcatattccggcgtggtggactgggcgaaaatgcgtgaaatcgctgacagcatcggtgcttacctgttcgttgatatggcgcacgttgcgggcctggttgctgctggcgtctacccgaacccggttcctcatgctcacgttgttactaccaccactcacaaaaccctggcgggtccgcgcggcggcctgatcctggcgaaaggtggtagcgaagagctgtacaaaaaactgaactctgccgttttccctggtggtcagggcggtccgttgatgcacgtaatcgccggtaaagcggttgctctgaaagaagcgatggagcctgagttcaaaacttaccagcagcaggtcgctaaaaacgctaaagcgatggtagaagtgttcctcgagcgcggctacaaagtggtttccggcggcactgataaccacctgttcctggttgatctggttgataaaaacctgaccggtaaagaagcagacgccgctctgggccgtgctaacatcaccgtcaacaaaaacagcgtaccgaacgatccgaagagcccgtttgtgacctccggtattcgtgtaggtactccggcgattacccgtcgcggctttaaagaagccgaagcgaaagaactggctggctggatgtgtgacgtgctggacagcatcaatgatgaagccgttatcgagcgcatcaaaggtaaagttctcgacatctgcgcacgttacccggtttacgcataacaattg

SEQ ID NO: 10 - DNA, 5784 bp, synthetic construct
  source 1..5784: mol_type = other DNA
tcatgagcttttttcacgccagccagcgggatgccctgaatcagagcctggcagaagtccaggggcagattaacgtttcgttcgagtttttcccgccgcgtaccagtgaaatggagcagaccctgtggaactccatcgatcgccttagcagcctgaaaccgaagtttgtatcggtgacctatggcgcgaactccggcgagcgcgaccgtacgcacagcattattaaaggcattaaagatcgcactggtctggaagcggcaccgcatcttacttgcattgatgcgacgcccgacgagctgcgcaccattgcacgcgactactggaataacggtattcgtcatatcgtggcgctgcgtggcgatctgccgccgggaagtggtaagccagaaatgtatgcttctgacctggtgacgctgttaaaagaagtggcagatttcgatatctccgtggcggcgtatccggaagttcacccggaagcaaaaagcgctcaggcggatttgcttaatctgaaacgcaaagtggatgccggagccaaccgcgcgattactcagttcttcttcgatgtcgaaagctacctgcgttttcgtgaccgctgtgtatcggcgggcattgatgtggaaattattccgggaattttgccggtatctaactttaaacaggcgaagaaatttgccgatatgaccaacgtgcgtattccggcgtggatggcgcaaatgttcgacggtctggatgatgatgccgaaacccgcaaactggttggcgcgaatattgccatggatatggtgaagattttaagccgtgaaggagtgaaagatttccacttctatacgcttaaccgtgctgaaatgagttacgcgatttgccatacgctgggggttcgacctggtttataagagctcaaagaggagaaaactagtatgagcagcaaagtggaacaactgcgtgcgcagttaaatgaacgtattctggtgctggacggcggtatgggcaccatgatccagagttatcgactgaacgaagccgattttcgtggtgaacgctttgccgactggccatgcgacctcaaaggcaacaacgacctgctggtactcagtaaaccggaagtgatcgccgctatccacaacgcctactttgaagcgggcgcggatatcatcgaaaccaacaccttcaactccacgaccattgcgatggcggattaccagatggaatccctgtcggcggaaatcaactttgcggcggcgaaactggcgcgagcttgtgctgacgagtggaccgcgcgcacgccagagaaaccgcgctacgttgccggtgttctcggcccgaccaaccgcacggcgtctatttctccggacgtcaacgatccggcatttcgtaatatcacttttgacgggctggtggcggcttatcgagagtccaccaaagcgctggtggaaggtggcgcggatctgatcctgattgaaaccgttttcgacacccttaacgccaaagcggcggtatttgcggtgaaaacggagtttgaagcgctgggcgttgagctgccgattatgatctccggcaccatcaccgacgcctccgggcgcacgctctccgggcagaccaccgaagcattttacaactcattgcgccacgccgaagctctgacctttggcctgaactgtgcgctggggcccgatgaactgcgccagtacgtgcaggagctgtcacggattgcggaatgctacgtcaccgcgcacccgaacgccgggctacccaacgcctttggtgagtacgatctcgacgccgacacgatggcaaaacagatacgtgaatgggcgcaagcgggttttctcaatatcgtcggcggctgctgtggcaccacgccacaacatattgcagcgatgagtcgtgcagtagaaggattagcgccgcgcaaactgccggaaattcccgtagcctgccgtttgtccggcctggagccgctgaacattggcgaagatagcctgtttgtgaacgtgggtgaacgcaccaacgtcaccggttccgctaagttcaagcgcctgatcaaagaagagaaatacagcgaggcgctggatgtcgcgcgtcaacaggtggaaaacggcgcgcagattatcgatatcaacatggatgaagggatgctcgatgccgaagcggcgatggtgcgttttctcaatctgattgccggtgaaccggatatcgctcgcgtgccgattatgatcgactcctcaaaatgggacgtcattgaaaaaggtctgaagtgtatccagggcaaaggcattgttaactctatctcgatgaaagagggcgtcgatgcctttatccatcacgcgaaattgttgcgtcgctacggtgcggcagtggtggtaatggcctttgacgaacagggacaggccgatactcgcgcacggaaaatcgagatttgccgtcgggcgtacaaaatcctcaccgaagaggttggcttcccgccagaagatatcatcttcgacccaaacatcttcgcggtcgcaactggcattgaagagcacaacaactacgcgcaggactttatcggcgcgtgtgaagacatcaaacgcgaactgccgcacgcgctgatttccggcggcgtatctaacgtttctttctcgttccgtggcaacgatccggtgcgcgaagccattcacgcagtgttcctctactacgctattcgcaatggcatggatatggggatcgtcaacgccgggcaactggcgatttacgacgacctacccgctgaactgcgcgacgcggtggaagatgtgattcttaatcgtcgcgacgatggcaccgagcgtttactggagcttgccgagaaatatcgcggcagcaaaaccgacgacaccgccaacgcccagcaggcggagtggcgctcgtgggaagtgaataaacgtctggaatactcgctggtcaaaggcattaccgagtttatcgagcaggataccgaagaagcccgccagcaggctacgcgcccgattgaagtgattgaaggcccgttgatggacggcatgaatgtggtcggcgacctgtttggcgaagggaaaatgttcctgccacaggtggtcaaatcggcgcgcgtcatgaaacaggcggtggcctacctcgaaccgtttattgaagccagcaaagagcagggcaaaaccaacggcaagatggtgatcgccaccgtgaagggcgacgtccacgacatcggtaaaaatatcgttggtgtggtgctgcaatgtaacaactacgaaattgtcgatctcggcgttatggtgcctgcggaaaaaattctccgtaccgctaaagaagtgaatgctgatctgattggcctttcggggcttatcacgccgtcgctggacgagatggttaacgtggcgaaagagatggagcgtcagggcttcactattccgttactgattggcggcgcgacgacctcaaaagcgcacacggcggtgaaaatcgagcagaactacagcggcccgacggtgtatgtgcagaatgcctcgcgtaccgttggtgtggtggcggcgctgctttccgatacccagcgtgatgattttgtcgctcgtacccgcaaggagtacgaaaccgtacgtattcagcacgggcgcaagaaaccgcgcacaccaccggtcacgctggaagcggcgcgcgataacgatttcgcttttgactggcaggcttacacgccgccggtggcgcaccgtctcggcgtgcaggaagtcgaagccagcatcgaaacgctgcgtaattacatcgactggacaccgttctttatgacctggtcgctggccgggaagtatccgcgcattctggaagatgaagtggtgggcgttgaggcgcagcggctgtttaaagacgccaacgacatgctggataaattaagcgccgagaaaacgctgaatccgcgtggcgtggtgggcctgttcccggcaaaccgtgtgggcgatgacattgaaatctaccgtgacgaaacgcgtacccatgtgatcaacgtcagccaccatctgcgtcaacagaccgaaaaaacaggcttcgctaactactgtctcgctgacttcgttgcgccgaagctttctggtaaagcagattacatcggcgcatttgccgtgactggcgggctggaagaggacgcactggctgatgcctttgaagcgcagcacgatgattacaacaaaatcatggtgaaagcgcttgccgaccgtttagccgaagcctttgcggagtatctccatgagcgtgtgcgtaaagtctactggggctatgcgccgaacgagaacctcagcaacgaagagctgatccgcgaaaactaccagggcatccgtccggcaccgggctatccggcctgcccggaacatacggaaaaagccaccatctgggagctgctggaagtggaaaaacacactggcatgaaactcacagaatctttcgccatgtggcccggtgcatcggtttcgggttggtacttcagccacccggacagcaagtactacgctgtagcacaaattcagcgcgatcaggttgaagattatgcccgccgtaaaggtatgagcgttaccgaagttgagcgctggctggcaccgaatctggggtatgacgcggactgactgcagagaggagaaaactagtatggcaaaacacctttttacgtccgagtccgtctctgaagggcatcctgacaaaattgctgaccaaatttctgatgccgttttagacgcgatcctcgaacaggatccgaaagcacgcgttgcttgcgaaacctacgtaaaaaccggcatggttttagttggcggcgaaatcaccaccagcgcctgggtagacatcgaagagatcacccgtaacaccgttcgcgaaattggctatgtgcattccgacatgggctttgacgctaactcctgtgcggttctgagcgctatcggcaaacagtctcctgacatcaaccagggcgttgaccgtgccgatccgctggaacagggcgcgggtgaccagggtctgatgtttggctacgcaactaatgaaaccgacgtgctgatgccagcacctatcacctatgcacaccgtctggtacagcgtcaggctgaagtgcgtaaaaacggcactctgccgtggctgcgcccggacgcgaaaagccaggtgacttttcagtatgacgacggcaaaatcgttggtatcgatgctgtcgtgctttccactcagcactctgaagagatcgaccagaaatcgctgcaagaagcggtaatggaagagatcatcaagccaattctgcccgctgaatggctgacttctgccaccaaattcttcatcaacccgaccggtcgtttcgttatcggtggcccaatgggtgactgcggtctgactggtcgtaaaattatcgttgatacctacggcggcatggcgcgtcacggtggcggtgcattctctggtaaagatccatcaaaagtggaccgttccgcagcctacgcagcacgttatgtcgcgaaaaacatcgttgctgctggcctggccgatcgttgtgaaattcaggtttcctacgcaatcggcgtggctgaaccgacctccatcatggtagaaactttcggtactgagaaagtgccttctgaacaactgaccctgctggtacgtgagttcttcgacctgcgcccatacggtctgattcagatgctggatctgctgcacccgatctacaaagaaaccgcagcatacggtcactttggtcgtgaacatttcccgtgggaaaaaaccgacaaagcgcagctgctgcgcgatgctgccggtctgaagtaagaattc

SEQ ID NO: 11 - DNA, 1045 bp, synthetic construct
  source 1..1045: mol_type = other DNA
ccatgggaagttcagaagatcaagcttataggttgctgaacgattacgcaaatggttttatggtcagccaagttctgtttgcggcgtgtgaacttggcgtattcgacctgttagccgaagcaccgggcccgctcgacgtggcagcggtggctgcgggtgttagagcgagcgcgcatggtactgagctgttgttggacatctgcgtttctctgaagctgctgaaggtggaaacccgaggtggcaaggcgttctatcgtaacaccgagctgtctagtgattacctgacgaccgtgtccccgaccagccagtgttccatgctcaagtacatgggtcgcacgagctatcgttgctggggtcatctggctgacgctgtccgtgaaggtcgcaaccagtatctggaaacctttggtgtgccggcagaggagctcttcaccgcgatctaccgcagcgaaggtgaacgtctccaattcatgcaggctctgcaagaggtttggtccgttaatggccgtagcgttctgactgccttcgacctatccgtgttcccgctgatgtgcgatctgggcggcggagccggtgcgctggcgaaagagtgcatgagcttgtacccaggctgcaaaatcacggtattcgacatcccggaagtcgtgtggaccgcgaagcagcacttcagctttcaagaagaggagcagattgatttccaagagggtgacttctttaaagatccgttaccggaggcagacctgtacattctggcccgtgttctgcacgattgggaagacggcaagtgcagccacctgttggagcgcatttaccacacctgtaaaccgggtggcggtattctggtgattgaaagccttctggacgaagatcgtcgtggcccattgctgacgcagctgtatagcctgaacatgttggttcagaccgagggccaggagcgcaccccgacccattatcacatgctgttgtcttcggctggttttcgtgactttcaatttaaaaaaaccggtgcgatctatgatgcgatcctcgctcgtaaataagatct

SEQ ID NO: 12 - DNA, 1266 bp, synthetic construct
  source 1..1266: mol_type = other DNA
caattgaaagaggagaaaactagtatgaaaatcggcatcattggtgcaatggaagaagaagttacgctgctgcgtgacaaaatcgaaaaccgtcaaactatcagtctcggcggttgcgaaatctataccggccaactgaatggaaccgaggttgcgcttctgaaatcgggcatcggtaaagtcgctgcggcgctgggtgccactttgctgttggaacactgcaagccagatgtgattattaacaccggttctgccggtggcctggcaccaacgttgaaagtgggcgatatcgttgtctcggacgaagcacgttatcacgacgcggatgtcacggcatttggttatgaatacggtcagttaccaggctgtccggcaggctttaaagctgacgataaactgatcgctgccgctgaggcctgcattgccgaactgaatcttaacgctgtacgtggcctgattgttagcggcgacgctttcatcaacggttctgttggtctggcgaaaatccgccacaacttcccacaggccattgctgtagagatggaagcgacggcaatcgcccatgtctgccacaatttcaacgtcccgtttgttgtcgtacgcgccatctccgacgtggccgatcaacagtctcatcttagcttcgatgagttcctggctgttgccgctaaacagtccagcctgatggttgagtcactggtgcagaaacttgcacatggctaaggtaccagaggagaaaactagtatgccgttgttagatagcttcacagtcgatcatacccggatggaagcgcctgcagttcgggtggcgaaaacaatgaacaccccgcatggcgacgcaatcaccgtgttcgatctgcgcttctgcgtgccgaacaaagaagtgatgccagaaagagggatccataccctggagcacctgtttgctggttttatgcgtaaccatcttaacggtaatggtgtagagattatcgatatctcgccaatgggctgccgcaccggtttttatatgagtctgattggtacgccagatgagcagcgtgttgctgatgcctggaaagcggcaatggaagacgtgctgaaagtgcaggatcagaatcagatcccggaactgaacgtctaccagtgtggcacttaccagatgcactcgttgcaggaagcgcaggatattgcgcgtagcattctggaacgtgacgtacgcatcaacagcaacgaagaactggcactgccgaaagagaagttgcaggaactgcacatctaggtacc

SEQ ID NO: 13 - DNA, 1550 bp, synthetic construct
  source 1..1550: mol_type = other DNA
ggtaccagaggagaaagacgtcatgcctgatatgaagctttttgctggtaacgccaccccggaactagcacaacgtattgccaaccgcctgtacacttcactcggcgacgccgctgtaggtcgctttagcgatggcgaagtcagcgtacaaattaatgaaaatgtacgcggtggtgatattttcatcatccagtccacttgtgcccctactaacgacaacctgatggaattagtcgttatggttgatgccctgcgtcgtgcttccgcaggtcgtatcaccgctgttatcccctactttggctatgcgcgccaggaccgtcgcgtccgttccgctcgtgtaccaatcactgcgaaagtggttgcagacttcctctccagcgtcggtgttgaccgtgtgctgacagtggatctgcacgctgaacagattcagggtttcttcgacgttccggttgataacgtatttggtagcccgatcctgctggaagacatgctgcagctgaatctggataacccaattgtggtttctccggacatcggcggcgttgtgcgtgcccgcgctatcgctaagctgctgaacgataccgatatggcaatcatcgacaaacgtcgtccgcgtgcgaacgtttcacaggtgatgcatatcatcggtgacgttgcaggtcgtgactgcgtactggtcgatgatatgatcgacactggcggtacgctgtgtaaagctgctgaagctctgaaagaacgtggtgctaaacgtgtatttgcgtacgcgactcacccgatcttctctggcaacgcggcgaacaacctgcgtaactctgtaattgatgaagtcgttgtctgcgataccattccgctgagcgatgaaatcaaatcactgccgaacgtgcgtactctgaccctgtcaggtatgctggccgaagcgattcgtcgtatcagcaacgaagaatcgatctctgccatgttcgaacactaagatctaaagaggagaaagacgtcatgaccgcgactgcacagcagcttgagtatctcaaaaatagcatcaaaagcattcaggactacccaaaacccggcattcttttccgcgatgtcaccagcttactggaagacccgaaagcttacgctctcagcatcgacttgctggttgagcgttacaaaaatgcgggcattaccaaagttgtcggcaccgaagcgcgtggcttcttgtttggcgctccggtagctctgggtctgggcgttggctttgtaccggtccgtaaaccgggcaaactgccgcgtgaaaccatcagtgaaacttacgacctggaatacggcaccgatcagctggagatccacgttgatgccatcaaaccgggcgacaaagttctggtggtggacgacctgctggcaaccggcggcactatcgaagcgaccgttaaactgatccgtcgtctgggtggtgaagtggctgacgctgcgttcattatcaacctgttcgatctcggcggcgaacagcgtctcgaaaaacagggcattaccagctacagccttgtcccgttcccgggccattaagatct